European Patent Application EP 4 729 533 A1, published April 22, 2026. Title: Fusion proteins comprising apolipoprotein or fragments thereof and uses thereof. Applicant: RNAGENE Inc. The sequence listing filed with the application follows.

SEQUENCE LISTING (11 sequences)

SEQ ID NO: 1 - protein, 299 aa, synthetic construct
KVEQAVETEPEPELRQQTEWQSGQRWELALGRFWDYLRWVQTLSEQVQEELLSSQVTQELRALMDETMKELKAYKSELEEQLTPVAEETRARLSKELQAAQARLGADMEDVCGRLVQYRGEVQAMLGQSTEELRVRLASHLRKLRKRLLRDADDLQKRLAVYQAGAREGAERGLSAIRERLGPLVEQGRVRAATVGSLAGQPLQERAQAWGERLRARMEEMGSRTRDRLDEVKEQVAEVRAKLEEQAQQIRLQAEAFQARLKSWFEPLVEDMQRQWAGLVEKVQAAVGTSAAPVPSDNH

SEQ ID NO: 2 - protein, 299 aa, synthetic construct
KVEQAVETEPEPELRQQTEWQSGQRWELALGRFWDYLRWVQTLSEQVQEELLSSQVTQELRALMDETMKELKAYKSELEEQLTPVAEETRARLSKELQAAQARLGADMEDVRGRLVQYRGEVQAMLGQSTEELRVRLASHLRKLRKRLLRDADDLQKRLAVYQAGAREGAERGLSAIRERLGPLVEQGRVRAATVGSLAGQPLQERAQAWGERLRARMEEMGSRTRDRLDEVKEQVAEVRAKLEEQAQQIRLQAEAFQARLKSWFEPLVEDMQRQWAGLVEKVQAAVGTSAAPVPSDNH

SEQ ID NO: 3 - protein, 149 aa, synthetic construct
DADDLQKRLAVYQAGAREGAERGLSAIRERLGPLVEQGRVRAATVGSLAGQPLQERAQAWGERLRARMEEMGSRTRDRLDEVKEQVAEVRAKLEEQAQQIRLQAEAFQARLKSWFEPLVEDMQRQWAGLVEKVQAAVGTSAAPVPSDNH

SEQ ID NO: 4 - protein, 94 aa, synthetic construct
RAQAWGERLRARMEEMGSRTRDRLDEVKEQVAEVRAKLEEQAQQIRLQAEAFQARLKSWFEPLVEDMQRQWAGLVEKVQAAVGTSAAPVPSDNH

SEQ ID NO: 5 - RNA, 897 nt, synthetic construct
  source 1..897: mol_type = other RNA
aaagtggagcaagctgtggaaacggagccagagcccgaattgcggcaacaaactgagtggcagagcggtcaaaggtgggaactcgcccttggtagattttgggattatttgcggtgggtccaaacactcagcgagcaggtacaagaggaactcctctcctcccaggttacacaggagctgagggctttgatggatgagacaatgaaggagctgaaggcttataaaagtgaattggaagaacagcttacgcctgttgctgaagagaccagagcaagactgagcaaggagcttcaagctgcccaggcacgacttggggccgacatggaagacgtttgtgggcgccttgtccaatacagaggagaggtgcaggcgatgctgggccagtctacagaggagctccgggttcggcttgcgtcacacctcagaaaattgaggaagcggctcctgcgcgatgctgacgatcttcagaaacgactggcagtatatcaggccggagcaagagagggtgccgaacgcgggttgagcgccatccgggaacgcttgggtccccttgttgaacaagggcgcgttagagccgcaaccgttgggagtttggctggtcagcctctccaggagcgagcgcaagcatggggtgagaggttgcgagcccggatggaggaaatgggatctaggacccgggaccgcctggatgaggttaaggaacaagtcgctgaggtacgcgcgaaacttgaggaacaagcacagcagattagacttcaggcagaggcatttcaggcgcggcttaagagttggttcgagccgctcgtggaagatatgcagcgccaatgggcaggactcgtcgaaaaagttcaggcagctgtcgggacgagtgcagcccctgtcccatcagacaatcac

SEQ ID NO: 6 - RNA, 897 nt, synthetic construct
  source 1..897: mol_type = other RNA
aaggtggagcaagcggtggagacagagccggagcccgagctgcgccagcagaccgagtggcagagcggccagcgctgggaactggcactgggtcgcttttgggattacctgcgctgggtgcagacactgtctgagcaggtgcaggaggagctgctcagctcccaggtcacccaggaactgagggcgctgatggacgagaccatgaaggagttgaaggcctacaaatcggaactggaggaacaactgaccccggtggcggaggagacgcgggcacggctgtccaaggagctgcaggcggcgcaggcccggctgggcgcggacatggaggacgtgtgcggccgcctggtgcagtaccgcggcgaggtgcaggccatgctcggccagagcaccgaggagctgcgggtgcgcctcgcctcccacctgcgcaagctgcgtaagcggctcctccgcgatgccgatgacctgcagaagcgcctggcagtgtaccaggccggggcccgcgagggcgccgagcgcggcctcagcgccatccgcgagcgcctggggcccctggtggaacagggccgcgtgcgggccgccactgtgggctccctggccggccagccgctacaggagcgggcccaggcctggggcgagcggctgcgcgcgcggatggaggagatgggcagccggacccgcgaccgcctggacgaggtgaaggagcaggtggcggaggtgcgcgccaagctggaggagcaggcccagcagatacgcctgcaggccgaggccttccaggcccgcctcaagagctggttcgagcccctggtggaagacatgcagcgccagtgggccgggctggtggagaaggtgcaggctgccgtgggcaccagcgccgcccctgtgcccagcgacaatcac

SEQ ID NO: 7 - RNA, 447 nt, synthetic construct
  source 1..447: mol_type = other RNA
gatgctgacgatcttcagaaacgactggcagtatatcaggccggagcaagagagggtgccgaacgcgggttgagcgccatccgggaacgcttgggtccccttgttgaacaagggcgcgttagagccgcaaccgttgggagtttggctggtcagcctctccaggagcgagcgcaagcatggggtgagaggttgcgagcccggatggaggaaatgggatctaggacccgggaccgcctggatgaggttaaggaacaagtcgctgaggtacgcgcgaaacttgaggaacaagcacagcagattagacttcaggcagaggcatttcaggcgcggcttaagagttggttcgagccgctcgtggaagatatgcagcgccaatgggcaggactcgtcgaaaaagttcaggcagctgtcgggacgagtgcagcccctgtcccatcagacaatcac

SEQ ID NO: 8 - RNA, 282 nt, synthetic construct
  source 1..282: mol_type = other RNA
cgagcgcaagcatggggtgagaggttgcgagcccggatggaggaaatgggatctaggacccgggaccgcctggatgaggttaaggaacaagtcgctgaggtacgcgcgaaacttgaggaacaagcacagcagattagacttcaggcagaggcatttcaggcgcggcttaagagttggttcgagccgctcgtggaagatatgcagcgccaatgggcaggactcgtcgaaaaagttcaggcagctgtcgggacgagtgcagcccctgtcccatcagacaatcac

SEQ ID NO: 9 - protein, 143 aa, synthetic construct
LEVPNGPWRSLTFYPAWLTVSEGANATFTCSLSNWSEDLMLNWNRLSPSNQTEKQAAFCNGLSQPVQDARFQIIQLPNRHDFHMNILDTRRNDSGIYLCGAISLHPKAKIEESPGAELVVTERILETSTRYPSPSPKPEGRFQ

SEQ ID NO: 10 - protein, 118 aa, synthetic construct
EEELQVIQPDKSVSVAAGESAILHCTVTSLIPVGPIQWFRGAGPARELIYNQKEGHFPRVTTVSESTKRENMDFSISISNITPADAGTYYCVKFRKGSPDTEFKSGAGTELSVRAKPS

SEQ ID NO: 11 - protein, 50 aa, synthetic construct
TSAEAAAKEAAAKEAAAKEAAAKALEAEAAAKEAAAKEAAAKEAAAKAGT